European Patent Application EP 4 407 039 A1, published July 31, 2024. Title: Method for producing saccharifying enzyme. Applicant: 花王株式会社. The sequence listing filed with the application follows.

SEQUENCE LISTING (53 sequences)

SEQ ID NO: 1 - DNA, 1089 bp, Aspergillus niger
  source 1..1089: mol_type = genomic DNA
  CDS 1..1089
atgcatttcctccagaacgccgttgtggccgccactatgggcgctgcgctggccgccgctgctcctctcgagaagcgctcctgcactttcacctccgcctctgctgccaagtccggcaagtcctcttgctccaccatcaccctcgacaacatcgcggtccccgctggtgagactcttgacttgactggcctcaagaagggtaccaccgtcatcttcgagggtgagaccaccttcggctacaaggaatggaagggtcccctgatctccatgtccggtaccgacatcaccgtcaagcaggcctccggtgccaagatcaactgcgacggtgctcgctggtgggacggcaagggtagcaacggtggcaagaccaagcccaagttcttccaggcccacaagctcgaccagtccagcatcaccggcctgaaggtctacaacacccctgtccagggtttcagcattctggccgaccacctgaccatcaccgatgtgaccatcgacaactccgccggtaccagcaagggtcacaacaccgatgcctttgacattggccagagtacctacatcaccattgacggtgccaccgtctacaaccaggatgactgcctggccatcaactcgggtgagcacatcaccttcaccaacggctactgtgatggtggccacggtctctccatcggttccatcggtggccgcagtgacaacaccgtcaacgacgtgaccatctccaactccaaggtgctcaactcccagaacggtgtccgcatcaagaccatctacggcaagactggcactgtcgagaacgtcaagtttgaggacatcaccctgtccgacatcagcaagtacggtattgtcgttgagcaggactacgagaacggcagccccaccggcacgcccaccaacggtgtcaaggttgaggacatcactttcaagaaggtcaccggcagcgtcaagagctctggtactgacatctacatcctgtgcggttccggcagctgctcgaactggacctggagcggtgttgatgtgactggcggcaagaagagcagcaagtgcaagaacgtcccctcgggcgcttcctgcagcgattaa

SEQ ID NO: 2 - protein, 362 aa, Aspergillus niger
MHFLQNAVVAATMGAALAAAAPLEKRSCTFTSASAAKSGKSSCSTITLDNIAVPAGETLDLTGLKKGTTVIFEGETTFGYKEWKGPLISMSGTDITVKQASGAKINCDGARWWDGKGSNGGKTKPKFFQAHKLDQSSITGLKVYNTPVQGFSILADHLTITDVTIDNSAGTSKGHNTDAFDIGQSTYITIDGATVYNQDDCLAINSGEHITFTNGYCDGGHGLSIGSIGGRSDNTVNDVTISNSKVLNSQNGVRIKTIYGKTGTVENVKFEDITLSDISKYGIVVEQDYENGSPTGTPTNGVKVEDITFKKVTGSVKSSGTDIYILCGSGSCSNWTWSGVDVTGGKKSSKCKNVPSGASCSD

SEQ ID NO: 3 - DNA, 1107 bp, Aspergillus niger
  source 1..1107: mol_type = genomic DNA
  CDS 1..1107
atgcactcttaccagcttcttggcctggccgctgtcggctccctcgtctctgccgcccccgctccttctcgcgtctccgagttcgctaagaaggcctctacctgcaccttcacctctgcctctgaggccagcgagagcatctccagctgctccgatgttgtcctgagcagcatcgaggtccccgctggcgagaccctggacctgtccgatgctgctgatggctccaccatcaccttcgagggcaccacttccttcggatacaaggaatggaagggtcccctgatccgcttcggtggtaaggatctgaccgtcaccatggccgacggcgctgtcatcgacggtgacggttcccgctggtgggacagcaagggtaccaacggtggcaagaccaagcccaagttcatgtacatccacgacgttgaggactcgaccttcaagggcatcaacatcaagaatactcccgtccaggccatcagtgtccaggctaccaacgtccacctgaacgacttcaccatcgacaactccgacggtgatgacaacggtggccacaacaccgacggtttcgacatcagcgagtccaccggtgtctacatcagcggtgctaccgtcaagaaccaggacgactgcattgccatcaactctggcgagagcatctctttcaccggcggtacctgctccggtggccacggtctctccatcggctctgtcggtggccgtgatgacaacaccgtcaagaacgtgaccatctccgactccactgtcagcaactccgccaatggtgtccgcatcaagaccatctacaaggagaccggcgatgtcagcgagatcacctactccaacatccagctctccggcatcaccgactacggtatcgtcatcgagcaggactacgagaacggctctcccaccggcaccccctccaccggtatccccatcactgatgtcactgttgacggtgtcaccggcactcttgaggatgacgccacccaggtctacattctctgcggtgacggctcttgctctgactggacctggtccggtgttgacctctctggtggcaagaccagcgataaatgcgagaacgttccttccggtgcttcttgctaa

SEQ ID NO: 4 - protein, 368 aa, Aspergillus niger
MHSYQLLGLAAVGSLVSAAPAPSRVSEFAKKASTCTFTSASEASESISSCSDVVLSSIEVPAGETLDLSDAADGSTITFEGTTSFGYKEWKGPLIRFGGKDLTVTMADGAVIDGDGSRWWDSKGTNGGKTKPKFMYIHDVEDSTFKGINIKNTPVQAISVQATNVHLNDFTIDNSDGDDNGGHNTDGFDISESTGVYISGATVKNQDDCIAINSGESISFTGGTCSGGHGLSIGSVGGRDDNTVKNVTISDSTVSNSANGVRIKTIYKETGDVSEITYSNIQLSGITDYGIVIEQDYENGSPTGTPSTGIPITDVTVDGVTGTLEDDATQVYILCGDGSCSDWTWSGVDLSGGKTSDKCENVPSGASC

SEQ ID NO: 5 - DNA, 1089 bp, Aspergillus niger
  source 1..1089: mol_type = genomic DNA
  CDS 1..1089
atgcactcgtttgcttctcttctcgcctacggcctggtcgccggcgccaccttcgcttctgcctctcctatcgaagctcgagacagctgcacgttcaccaccgctgccgctgctaaagcgggcaaggcgaaatgctctactatcacccttaacaacatcgaagttccagctggaaccaccctcgacctgaccggtctcaccagcggtaccaaggtcatcttcgagggcaccacgaccttccagtacgaagaatgggcaggccccttgatctccatgagtggcgaacatatcaccgtcactggtgcctccggccacctcatcaattgcgatggtgcgcgctggtgggatggcaagggaaccagcggaaagaagaagcccaagttcttttacgcccatggccttgactcctcgtctattactggattaaacatcaaaaacactccccttatggcgtttagtgtccaggcgaatgacattacgtttaccgatgttaccatcaataatgcggatggcgacacccagggtggacacaacactgatgcgttcgatgttggtaactcggtcggggtgaatatcattaagccttgggtccataaccaggatgactgtcttgcgattaactctggcgagaacatctggttcaccggcggcacctgcattggcggccacggtctctccatcggctctgtcggcgaccgctccaacaacgtcgtcaagaacgtcaccatcgaacactccaccgtgagcaattccgaaaacgccgtccgaatcaagaccatctctggcgccactggctccgtgtctgagattacatactccaacatcgtcatgtccggcatctccgattacggcgtggtcattcagcaggattacgaagacggcaagcctacgggtaagccgacgaacggtgtcactattcaggatgtcaagctggagagcgtgaccggtagcgtggatagtaaggctactgagatctatcttctttgcgggtctggtagctgctcggactggacctgggacgatgtgaaggttactggggggaagaagtccaccgcttgcaagaacttcccttcggtggcctcttgctag

SEQ ID NO: 6 - protein, 362 aa, Aspergillus niger
MHSFASLLAYGLVAGATFASASPIEARDSCTFTTAAAAKAGKAKCSTITLNNIEVPAGTTLDLTGLTSGTKVIFEGTTTFQYEEWAGPLISMSGEHITVTGASGHLINCDGARWWDGKGTSGKKKPKFFYAHGLDSSSITGLNIKNTPLMAFSVQANDITFTDVTINNADGDTQGGHNTDAFDVGNSVGVNIIKPWVHNQDDCLAINSGENIWFTGGTCIGGHGLSIGSVGDRSNNVVKNVTIEHSTVSNSENAVRIKTISGATGSVSEITYSNIVMSGISDYGVVIQQDYEDGKPTGKPTNGVTIQDVKLESVTGSVDSKATEIYLLCGSGSCSDWTWDDVKVTGGKKSTACKNFPSVASC

SEQ ID NO: 7 - DNA, 1122 bp, Aspergillus niger
  source 1..1122: mol_type = genomic DNA
  CDS 1..1122
atgaagtacgctgctgctctcacggctgttgccgccctcgctgcccgcgccgctgctgtcggtgtctccggcactcccgtgggtttcgcctcctccgccactggtggtggtgatgctacccccgtctaccctaccaccaccgatgagctggtctcttacctcggtgatgacgaggcccgtgtcattgtcctgtccaagactttcgacttcactgacactgagggcactaccacgaccaccggttgcgctccctggggtactgcctccggctgccagctggccatcaacaaggacgactggtgcaccaactacgagcccgatgctcccaccaccaccgtcacctacaacactgctggtgaactcggtatcaccgtcaactccaacaagtccttgatcggtgagggtaccagcggtgtcatcaagggccgtggtctccgcatggtcagcggtgtctccaacatcatcatccagaacattgctgtcaccgacatcaaccccgagtacgtctggggtggtgacgccatcaccctcgacgaggctgacttggtctggattgaccacgttaccactgcccgcattggtcgccagcactacgtcctcggtaccgacgccgacagccgtgtctccatcaccaacaactacatcaacggcgagtctgactactctgctacttgcgacggccaccactactggaacgtgtaccttgacggctctagcgacaaggtcaccttcagtggcaactacctgtacaagacctccggccgtgcccccaaggtccaggacaacacctacctccacatctacaacaactactgggagaacaactcgggccacgctttcgagatcggctccggtggctacgtcctcgccgagggtaactacttctccaacgtcgacaccgtcctcgagaccgacaccttcgagggtgctctcttctcctctgacagcgcctcctccacctgcgagtcctacattggccgttcctgcgttgccaacgtcaacggcggtgacctcaccggcacctccaccaccgtcctctccaacctcagcggcgacaccctcccctctgctgatgctgccagcaccagccccgcctccaacgctggtcagggtaacctgtaa

SEQ ID NO: 8 - protein, 373 aa, Aspergillus niger
MKYAAALTAVAALAARAAAVGVSGTPVGFASSATGGGDATPVYPTTTDELVSYLGDDEARVIVLSKTFDFTDTEGTTTTTGCAPWGTASGCQLAINKDDWCTNYEPDAPTTTVTYNTAGELGITVNSNKSLIGEGTSGVIKGRGLRMVSGVSNIIIQNIAVTDINPEYVWGGDAITLDEADLVWIDHVTTARIGRQHYVLGTDADSRVSITNNYINGESDYSATCDGHHYWNVYLDGSSDKVTFSGNYLYKTSGRAPKVQDNTYLHIYNNYWENNSGHAFEIGSGGYVLAEGNYFSNVDTVLETDTFEGALFSSDSASSTCESYIGRSCVANVNGGDLTGTSTTVLSNLSGDTLPSADAASTSPASNAGQGNL

SEQ ID NO: 9 - DNA, 1140 bp, Aspergillus niger
  source 1..1140: mol_type = genomic DNA
  CDS 1..1140
atgaagtactctactatcttcagcgctgctgccgctgttttcgctggttccgccgctgcagtcggcgtgtccggctctgctgagggtttcgccgagggcgtcaccggtggcggtgatgccacccccgtctaccccgacactatcgatgagctggtctcttaccttggagacgatgaggcccgcgtcattgtcctgaccaagaccttcgacttcaccgacagcgaaggtaccaccactggcactggttgcgctccctggggtaccgcttccgcctgccaggttgctattgaccaggacgactggtgcgagaactacgagcccgatgctccctctatcagcgttgaatactacaacgctggtgtcctcggtatcaccgtcacctccaacaagtccctcatcggtgagggctcctctggtgcaatcaagggcaagggtctccgtattgtcagcggtgctgagaacatcatcatccagaacatcgcggttaccgacatcaaccccaagtacgtctggggtggtgatgctattactcttgatgactgcgacctggtctggatcgaccatgttactaccgcccgcatcggtcgccagcactacgtccttggaaccagcgccgacaaccgcgtctctctcaccaacaactacattgacggtgtctccgactactccgccacctgcgatggctaccactactggggcatctacctcgatggtgacgccgacttggtcaccatgaagggcaactacatctaccacacctccggccgtagccccaaggtccaggacaacactctcctccactgtgtcaacaactacttctacgacatctccggccacgcttttgagatcggtgagggtggctacgtcctggctgagggcaacgttttccagaacgtcgacaccgtccttgagacctacgagggcgcggccttcaccgtcccctccaccaccgccggtgaagtctgctccacctaccttggccgtgactgtgtcatcaacggcttcggctcctccggcactttctccgaggacagcacctctttcctctccgacttcgagggcaagaacattgcctctgcttccgcttacacctctgttgcctctagcgttgttgctaacgccggtcagggcaacctgtaa

SEQ ID NO: 10 - protein, 379 aa, Aspergillus niger
MKYSTIFSAAAAVFAGSAAAVGVSGSAEGFAEGVTGGGDATPVYPDTIDELVSYLGDDEARVIVLTKTFDFTDSEGTTTGTGCAPWGTASACQVAIDQDDWCENYEPDAPSISVEYYNAGVLGITVTSNKSLIGEGSSGAIKGKGLRIVSGAENIIIQNIAVTDINPKYVWGGDAITLDDCDLVWIDHVTTARIGRQHYVLGTSADNRVSLTNNYIDGVSDYSATCDGYHYWGIYLDGDADLVTMKGNYIYHTSGRSPKVQDNTLLHCVNNYFYDISGHAFEIGEGGYVLAEGNVFQNVDTVLETYEGAAFTVPSTTAGEVCSTYLGRDCVINGFGSSGTFSEDSTSFLSDFEGKNIASASAYTSVASSVVANAGQGNL

SEQ ID NO: 11 - DNA, 3821 bp, Trichoderma reesei
  source 1..3821: mol_type = genomic DNA
aattacaagtctcctctttctaccccctcctctcccccctctcctctgcttatttcataaccatctcctgtttcgccatttaaacgtacattcaaagctctctcggcgccgtctgcccacacatcaacaagcatcacgcctgcagcagcatctctaggactgctcgcgcctgaaaagcagatcaacaagagcagttcagactggcattctatccggccctattctcattccgacggttactctgccaccgaccgtgcccagaaggaataccagaacacctgaacctgctggaaggcaccttttagtccaccaactttggaacgacgcagcctcttctctcaaagctcagatcatagacgcagccagcgacatgcagtgcaatgtcatggatgttttgtgggttacgttcgtccctacagagtcactggcaggctacatgcatgtcatggtcccatatcgcccattcgaccaccgtcagcccagtacttgctcgtgtcaatctccgtcagtcgcgtgtgatcagacattccaactggatctgggccagccgggcactctttgccttgtcctgtttgacaggttcaatttgctctgtatgccacttctgtccagtctgtttagtgagccagactgctgagacactctgaaccgaggagcaagcgcctccacagccaagaagttgaagaagacggcagacacccacacagtgaccacgaagctttgtcacgcagtattgatcccatcaaccactagcaaatccctagacaccccgaaaggacttcaacagtgacctagcagcaaagccgtgagtctcggacggcctcttgttcaactcaaccgaccttccaagctacaaaaacgacaaggttggatgtctgccgtttgctgcctcgccaccagctgactttaggcaaaacaggtcattgaatccagatcggagtcgacactcgcatccgtgctccgggagtcacgatcgagacatgccgcccaagcatgcaacctgccccagggtccgattatatccaatttagccgctggacaagctgcatccatgccgctcatcacccccgcaaatcactttcgggtcccgtcttctcccagattgctttcatcggcactagaccaatggagagcggctcttgctgaatgccgtcgtaggctgttgtcgacggacctcggggtgcatgaggctgggaacagggggtgggggacatggcatggtgtgtgtgtgtgttatggttaattggaagcatacgggttgactctacttggttataacggccacattcgacatcaggtaatggatgtgacatggccgctccacggcgggctttgggcgtgaattacgacattgcggcaaagatggaatggactattcgccattctagcacgcgatattgtgatgctgctgctgatggctaatcccaaagactcgtcatactgcctcttgtagtttactgcatcgtcttgactccactgagaggactgtgccgatgagacgctgctgagaaacgtcgaatcggttgtacactcggagcattttggggtaacttgttgattttccatttccttctatacgtccatgagtttccgttccgatatatgagattgccaagaggaaattagccgttattcagacaatgtatgtgccgggcttcttctcacatgtatcggagcagaaggggtccatctatgtgagctgactcgagacggctgagacagcagcatcaccacgtcacgatggtgttgcaaggcgcaatatcattgatgaaaggagaacaacttctagactgggtaaattggtcaatggccagccgctcggccgtgcggagacgaggcaagcttgatgaggccaaattatccgtcaactgtcttataaaggagcccatgccaaaccccccctaaagactcaagaagccaaacctgaacaaccccagcacctgaacagtcatacaacccctccaagcccaaaagacacaacaactcctactagctgaagcaagaagacatcaacatggtctccttcacctccctcctcgccggcgtcgccgccatctcgggcgtcttggccgctcccgccgccgaggtcgaatccgtggctgtggagaagcgccagacgattcagcccggcacgggctacaacaacggctacttctactcgtactggaacgatggccacggcggcgtgacgtacaccaatggtcccggcgggcagttctccgtcaactggtccaactcgggcaactttgtcggcggcaagggatggcagcccggcaccaagaacaagtaagactacctactcttaccccctttgaccaacacagcacaacacaatacaacacatgtgactaccaatcatggaatcggatctaacagctgtgttttcaaaaaaaagggtcatcaacttctcgggcagctacaaccccaacggcaacagctacctctccgtgtacggctggtcccgcaaccccctgatcgagtactacatcgtcgagaactttggcacctacaacccgtccacgggcgccaccaagctgggcgaggtcacctccgacggcagcgtctacgacatttaccgcacgcagcgcgtcaaccagccgtccatcatcggcaccgccaccttttaccagtactggtccgtccgccgcaaccaccgctcgagcggctccgtcaacacggcgaaccacttcaacgcgtgggctcagcaaggcctgacgctcgggacgatggattaccagattgttgccgtggagggttactttagctctggctctgcttccatcaccgtcagctaaagggggctcttcttttgtgatgtgtgaaaaaaaaaaaaaggatggtggataaaagggggttgaagggcttgtgttctttggctctgtagaggctctagggggttggattgggctgactatggtctcccctttgtatgctacacactgatcagacgatcgtagtcagttgagagatgagcttcattggtcgatatgagtgctttgagactggacacttgcgtgactgcatgttccgtttcttgtgataattgccgtgaagatgtgtctgctggtatgacgacaaagtagcatcagcagcaaagtatggcgaggactactaggcccaagatattgtcggcttcgtcaaagtgagaaattttagggtctccattgattacattcatccgtttcagaagcacgatatagaggagtagcaccatcaggtcggaaaggtcgtcaacagcttgaacaagtcatactaaggtatgttagtgtggtcgtggttgtcggtatcagtaggtatcattggagtatgtgttatatacagattaatgggaccaatgcatcacgcatcaggacatgccctggcaatcctccctcttacaaatcgcgatgaggcttgggtttgggggtaatagtagcggtcgtaaaggtggtggtgccagtagcgcacacgcagccctggccggaaatgctggtaatgggaggagatttgcaggtgggctcggtggtaaaggaggcgtaggtgctggtgggctcaaccgtgggctcaaccagctcagccttgaccaggacggggatgatctggcctgtggacaggctgaaggagcggtggttgagcacggtgagaatggcgccaatctcgcccgagtggctggtgatgctaatccaggtgttgtcgtcgtgcgaaaagacgtcgtcaatcgcctccttggaacgggcgacctggtgagcaggcgtctcgccctcgtcctctttgccgcgccacagcaggtcctcctcggtgaagccagcctcgaactcaaagttgggagcgtaggcgtgaat

SEQ ID NO: 12 - DNA, 35 bp, synthetic construct
  source 1..35: mol_type = other DNA
gacaacgtagccgagctcttcttttgtgatgtgtg

SEQ ID NO: 13 - DNA, 35 bp, synthetic construct
  source 1..35: mol_type = other DNA
tttcgccacggagctttagctgacggtgatggaag

SEQ ID NO: 14 - DNA, 20 bp, synthetic construct
  source 1..20: mol_type = other DNA
agctccgtggcgaaagcctg

SEQ ID NO: 15 - DNA, 20 bp, synthetic construct
  source 1..20: mol_type = other DNA
ctcggctacgttgtcatcgt

SEQ ID NO: 16 - DNA, 35 bp, synthetic construct
  source 1..35: mol_type = other DNA
atatctggtggatctctcttcttttgtgatgtgtg

SEQ ID NO: 17 - DNA, 35 bp, synthetic construct
  source 1..35: mol_type = other DNA
acaacgagaaaagaactcggctacgttgtcatcgt

SEQ ID NO: 18 - DNA, 20 bp, synthetic construct
  source 1..20: mol_type = other DNA
ttcttttctcgttgtctcac

SEQ ID NO: 19 - DNA, 20 bp, synthetic construct
  source 1..20: mol_type = other DNA
agatccaccagatatgtcag

SEQ ID NO: 20 - DNA, 20 bp, synthetic construct
  source 1..20: mol_type = other DNA
ttcttttctcgttgtctcac

SEQ ID NO: 21 - DNA, 22 bp, synthetic construct
  source 1..22: mol_type = other DNA
ctcggctacgttgtcatcgtct

SEQ ID NO: 22 - DNA, 35 bp, synthetic construct; identical to SEQ ID NO: 12
  source 1..35: mol_type = other DNA

SEQ ID NO: 23 - DNA, 35 bp, synthetic construct
  source 1..35: mol_type = other DNA
acaacgagaaaagaaaatgatacctactgataccg

SEQ ID NO: 24 - DNA, 20 bp, synthetic construct
  source 1..20: mol_type = other DNA
taaagctccgtggcgaaagc

SEQ ID NO: 25 - DNA, 20 bp, synthetic construct
  source 1..20: mol_type = other DNA
gttgatgtcttcttgcttca

SEQ ID NO: 26 - DNA, 35 bp, synthetic construct
  source 1..35: mol_type = other DNA
caagaagacatcaacatgcactcttaccagcttct

SEQ ID NO: 27 - DNA, 35 bp, synthetic construct
  source 1..35: mol_type = other DNA
cgccacggagctttagcaagaagcaccggaaggaa

SEQ ID NO: 28 - DNA, 35 bp, synthetic construct
  source 1..35: mol_type = other DNA
caagaagacatcaacatgcactcgtttgcttctct

SEQ ID NO: 29 - DNA, 35 bp, synthetic construct
  source 1..35: mol_type = other DNA
cgccacggagctttaacaagaggccaccgaaggga

SEQ ID NO: 30 - DNA, 35 bp, synthetic construct
  source 1..35: mol_type = other DNA
caagaagacatcaacatgcatttcctccagaacgc

SEQ ID NO: 31 - DNA, 35 bp, synthetic construct
  source 1..35: mol_type = other DNA
cgccacggagctttaatcgctgcaggaagcgcccg

SEQ ID NO: 32 - DNA, 35 bp, synthetic construct
  source 1..35: mol_type = other DNA
caagaagacatcaacatgaagtacgctgctgctct

SEQ ID NO: 33 - DNA, 35 bp, synthetic construct
  source 1..35: mol_type = other DNA
cgccacggagctttacaggttaccctgaccagcgt

SEQ ID NO: 34 - DNA, 35 bp, synthetic construct
  source 1..35: mol_type = other DNA
caagaagacatcaacatgaagtactctactatctt

SEQ ID NO: 35 - DNA, 35 bp, synthetic construct
  source 1..35: mol_type = other DNA
cgccacggagctttacaggttgccctgaccggcgt

SEQ ID NO: 36 - DNA, 1266 bp, Aspergillus niger
  source 1..1266: mol_type = genomic DNA
gttccacactccagcagagcatctcggagccaacaatgcgtggttccgtccaaataccaggcatcgaatgggacggctgatgactcggctgctgtctcccaggcctttgcacaatgcgcgactgactcggttattattttcgaggagggtgtcaactataacatctttcagccgatcaccgccaccaacctcagcaatgtggaaatccggatgcacggcaacctgcatctgccacagaatatcactgcggtgcagaatatagtcagtgacggtacttctacatggtttaccctagaaggaccaaaagtggactggattggtcctgaagacgtgaacaatggttggattgactcgtacggacaaccgtggtgggatgcgaaccctgcaggtagttcaggcatcgataaccgtccgcatctcatgagcttcaagtctagccaagccactatgaaatacttcaggtctaggaagcccatcgcctggaatgtcaaactgcatggacaagacattacagtcagccacgctattatcgacgctacctcgacaggtagcttcccattcaacactgacggtttcgatgttgagggtaccaatatccagatcaccgacagtatcatgtacaacggcgacgatgcgattgcagtaggcgcggactcgcacgacatacttttcacaagaaacaccatcggctaccagactcacggcatgagcattggatcgctgggaaaggatcccacagacttcgccaatatcagcaacatccgctttgacgatgtgactgttgtcgatgggctctacgcagcacgcttcaagtcatggagcggagggaccggactcgtcaagaatgtgacctggaacaatattagagtcttcaacgtgacgttcccgatctttgtgactcagagttatagcgaccaaggcgcctcccggtctggaactgtcaatgctagttcggctgtgatgatggaggattttacctggtctgactttgctggctcgatcaatacgtaccagcctggtgacggttcttgcgtttccgacccttgctggtacaacgttgggctgccaaatttgaagcatacggaggccctcattatcgaatgccatactgctcaatcttgtaagaactttgtgacggacaacatccagctatacccgcaggttctggaaccagcgagtgtgatctgcatgaacgcaacggcagccctcaatcctgatcttggatttacatgtaaaaacgggacctacagcccattatctaattaa

SEQ ID NO: 37 - protein, 421 aa, Aspergillus niger
VPHSSRASRSQQCVVPSKYQASNGTADDSAAVSQAFAQCATDSVIIFEEGVNYNIFQPITATNLSNVEIRMHGNLHLPQNITAVQNIVSDGTSTWFTLEGPKVDWIGPEDVNNGWIDSYGQPWWDANPAGSSGIDNRPHLMSFKSSQATMKYFRSRKPIAWNVKLHGQDITVSHAIIDATSTGSFPFNTDGFDVEGTNIQITDSIMYNGDDAIAVGADSHDILFTRNTIGYQTHGMSIGSLGKDPTDFANISNIRFDDVTVVDGLYAARFKSWSGGTGLVKNVTWNNIRVFNVTFPIFVTQSYSDQGASRSGTVNASSAVMMEDFTWSDFAGSINTYQPGDGSCVSDPCWYNVGLPNLKHTEALIIECHTAQSCKNFVTDNIQLYPQVLEPASVICMNATAALNPDLGFTCKNGTYSPLSN

SEQ ID NO: 38 - DNA, 1212 bp, Aspergillus niger
  source 1..1212: mol_type = genomic DNA
ggtaatgtggaaaacaaccacaatgtctgcaccgtccgagcaaacgggggacaccaagatgacgtccccaatattatggcggcgttcaaagagtgtggcaatggaggtaccattattttccccgaagaccaatcgtactggattgcgacgagactgcatcccacattgaaggacgtcgcaatcgaatggcgggggaagtggacattttccgacaacctcacctactggcgtaacaactcctaccccattgcgttccagaaccatcatgccggcttcattattagcggcgacaacatcaccatcaatggctatggcaccggcggcattgatggcaatggcaatacttggtacacagccgagaagggcgacacgcagccggggcgtccgatgccatttgtcttttggaacgtgtctgaggttattgttgacagtttctacgtcaaggatccgcccctctggagtgtcaacatcatgaacgggactaacatgcgtttcaacaatatctactgcaacgccacggctgtagatgccccctggggcgataactgggtgcagaatacggatggtttcgataccatggacgctaccaacatccagctcaccaacttcgtctaccaaggcggagatgactgcatcgctatcaagccccgctcctacaacatcgacatccagaatgttacctgccgtggaggcaacggcattgccattggcagcttgggtcaatatttggaagatagcagtgttgctaacattcgcgtggacaaggtcaatatcatccgctacaacgaagacatgcacaacagcgcctacctcaagacctgggtcggagctctcgtcccccaaagttcctacgaaagcgccggcgtacctcgtggcgatggctggggcagcatccgtaacgtcctattttcaaacttcaatgtacaaggcgcaagcgctggcccttccatcagtcaggacagtggagacaacggttcctatgcgggtacaagcaagatgtctatttcaaatgttgcgtttgtcaatttcacgggatgggtggatactgagaagtctgtggtctcgacggtctcctgctcagaggtacatccgtgctacaatatcgactatgacaatgtggtgttgtatccagggaagaatgccacaacagctgggacagggtcttgtaaatatacagctgatggaggagtgcatgggttgagtgggtgttga

SEQ ID NO: 39 - protein, 403 aa, Aspergillus niger
GNVENNHNVCTVRANGGHQDDVPNIMAAFKECGNGGTIIFPEDQSYWIATRLHPTLKDVAIEWRGKWTFSDNLTYWRNNSYPIAFQNHHAGFIISGDNITINGYGTGGIDGNGNTWYTAEKGDTQPGRPMPFVFWNVSEVIVDSFYVKDPPLWSVNIMNGTNMRFNNIYCNATAVDAPWGDNWVQNTDGFDTMDATNIQLTNFVYQGGDDCIAIKPRSYNIDIQNVTCRGGNGIAIGSLGQYLEDSSVANIRVDKVNIIRYNEDMHNSAYLKTWVGALVPQSSYESAGVPRGDGWGSIRNVLFSNFNVQGASAGPSISQDSGDNGSYAGTSKMSISNVAFVNFTGWVDTEKSVVSTVSCSEVHPCYNIDYDNVVLYPGKNATTAGTGSCKYTADGGVHGLSGC

SEQ ID NO: 40 - DNA, 1314 bp, Fusarium oxysporum
  source 1..1314: mol_type = genomic DNA
gtggttggtacttcttcccgcaattccgccctgccgaaacgtccccatgtcgaagctgctccatatggcactggcaaggcctttccggctagtcctgctcgatctcgcaaggacttctgctacgtcaaccccgggaagggcaagaacgttgacgatgcgccctctatcctgaaggcctttaagaagtgcaacaaaggtggcacgattgtcctcgatcagaagtactccattgcatcgcctttggacctgacctggcttgcccacgttgacgtgattatcaccggcgaggtgaacttcaagtcagacccctactactgggccgatcacagcttcaagtacgatttccagaacatgagcagcttttggaagatcggtggcaaggacatccacatctacggcgacctcaccaagggagagtcgctcctggatggccacggtcaagcgtactgggaagagatggccgtcaacaagacactccttaggccgattctcctcacgatcgaagacgcccacggactgaccatgagcaacctgcgtatgcgcaatccacccaactggttcaacatcatcatcaactccacggatgtgctgatttcagacctagatctcgaggcgaagtccctcaatggcgtcaagattgccaacagtgatggctgggacacctatcgctcggacagaatcgtcatccagaattccgtgatcgacaacaccgacgactgcgtctcctttaagcccaacagcacaaacgtggtcgtccaaaacctcgtctgcaatggctcgcatggcatcagcgtcggatccctggggcagtataagggcgagactgacatagtcgagaacctgtacatctacaacatctcgatgtccaatgcctctgatggcgctaggattaaggtgtggcctggggttgagacggccttccagtccctccttaacggaggcggcggtttgggacgagtgcggaacgtcacgtacgacaccttctaccacgagaacaacgacaacgccatcaccattacccagtgctatggccagaagaaccagaccctctgcaacgagttccccgccaacctcacgattgaggacgtcacgatgaagaacttttggggcacagtctcgaccaagtacgaccctcgagcgggctctttggtctgtagcgcaccggaccgctgcagcaatattgtcgctgaggatatcaaggtccaagtccccagcaaaaagcctcccgtctacgactgccagaacatcgacacctcgactctggacatcacgtgtcgcgacccaactaacgcacgggacaccacaaacggctaa

SEQ ID NO: 41 - protein, 437 aa, Fusarium oxysporum
VVGTSSRNSALPKRPHVEAAPYGTGKAFPASPARSRKDFCYVNPGKGKNVDDAPSILKAFKKCNKGGTIVLDQKYSIASPLDLTWLAHVDVIITGEVNFKSDPYYWADHSFKYDFQNMSSFWKIGGKDIHIYGDLTKGESLLDGHGQAYWEEMAVNKTLLRPILLTIEDAHGLTMSNLRMRNPPNWFNIIINSTDVLISDLDLEAKSLNGVKIANSDGWDTYRSDRIVIQNSVIDNTDDCVSFKPNSTNVVVQNLVCNGSHGISVGSLGQYKGETDIVENLYIYNISMSNASDGARIKVWPGVETAFQSLLNGGGGLGRVRNVTYDTFYHENNDNAITITQCYGQKNQTLCNEFPANLTIEDVTMKNFWGTVSTKYDPRAGSLVCSAPDRCSNIVAEDIKVQVPSKKPPVYDCQNIDTSTLDITCRDPTNARDTTNG

SEQ ID NO: 42 - DNA, 22 bp, synthetic construct
  source 1..22: mol_type = other DNA
taaaggggcggccgctcaagag

SEQ ID NO: 43 - DNA, 20 bp, synthetic construct
  source 1..20: mol_type = other DNA
agcttcggcctctcttttct

SEQ ID NO: 44 - DNA, 35 bp, synthetic construct
  source 1..35: mol_type = other DNA
agagaggccgaagctgttccacactccagcagagc

SEQ ID NO: 45 - DNA, 35 bp, synthetic construct
  source 1..35: mol_type = other DNA
gcggccgcccctttattaattagataatgggctgt

SEQ ID NO: 46 - DNA, 35 bp, synthetic construct
  source 1..35: mol_type = other DNA
agagaggccgaagctggtaatgtggaaaacaacca

SEQ ID NO: 47 - DNA, 35 bp, synthetic construct
  source 1..35: mol_type = other DNA
gcggccgcccctttatcaacacccactcaacccat

SEQ ID NO: 48 - DNA, 35 bp, synthetic construct
  source 1..35: mol_type = other DNA
agagaggccgaagctgtggttggtacttcttcccg

SEQ ID NO: 49 - DNA, 35 bp, synthetic construct
  source 1..35: mol_type = other DNA
gcggccgcccctttattagccgtttgtggtgtccc

SEQ ID NO: 50 - DNA, 35 bp, synthetic construct
  source 1..35: mol_type = other DNA
agagaggccgaagctgctcctctcgagaagcgctc

SEQ ID NO: 51 - DNA, 35 bp, synthetic construct
  source 1..35: mol_type = other DNA
gcggccgcccctttattaatcgctgcaggaagcgc

SEQ ID NO: 52 - DNA, 35 bp, synthetic construct
  source 1..35: mol_type = other DNA
agagaggccgaagctgtcggtgtctccggcactcc

SEQ ID NO: 53 - DNA, 35 bp, synthetic construct
  source 1..35: mol_type = other DNA
gcggccgcccctttattacaggttaccctgaccag